European Patent Specification EP 4 301 770 B1, published August 27, 2025. Title: LONG ACTING AMYLIN RECEPTOR AGONISTS AND USES THEREOF. Applicant: Eli Lilly and Company. The sequence listing filed with the application follows.

SEQUENCE LISTING (25 sequences)

SEQ ID NO: 1 - protein, 37 aa, Artificial Sequence
  Synthetic Construct
  MISC_FEATURE (1)..(1): Xaa at position 1 is gamma-Glu
  MISC_FEATURE (11)..(11): Xaa at position 11 is Orn
  MISC_FEATURE (15)..(15): Xaa at position 15 is alpha-methyl-Phe
  MISC_FEATURE (22)..(22): Xaa at position 22 is N-methyl-Asn
  MOD_RES (37)..(37): Tyr at position 37 is amidated
XCNTATCATGXLAEXLVRSSNXFGPKLPPTEVGSNTY

SEQ ID NO: 2 - protein, 37 aa, Artificial Sequence; identical to SEQ ID NO: 1
  Synthetic Construct
  MISC_FEATURE (1)..(1): Xaa at position 1 is gamma-Glu
  MOD_RES (2)..(7): There is a thioacetal bridge between the cysteines at positions 2 and 7
  MISC_FEATURE (11)..(11): Xaa at position 11 is Orn
  MISC_FEATURE (15)..(15): Xaa at position 15 is alpha-methyl-Phe
  MISC_FEATURE (22)..(22): Xaa at position 22 is N-methyl-Asn
  MOD_RES (26)..(26): The lysine at position 26 is attached to a fatty acid linker moiety according to the formula (gamma-Glu)2-CO-(CH2)18-CO2H
  MOD_RES (37)..(37): Tyr at position 37 is amidated

SEQ ID NO: 3 - protein, 37 aa, Artificial Sequence; identical to SEQ ID NO: 1
  Synthetic Construct
  MISC_FEATURE (1)..(1): Xaa at position 1 is gamma-Glu
  MISC_FEATURE (11)..(11): Xaa at position 11 is Orn
  MISC_FEATURE (15)..(15): Xaa at position 15 is alpha-methyl-Phe
  MISC_FEATURE (22)..(22): Xaa at position 22 is N-methyl-Asp
  MOD_RES (37)..(37): Tyr at position 37 is amidated

SEQ ID NO: 4 - protein, 37 aa, Artificial Sequence; identical to SEQ ID NO: 1
  Synthetic Construct
  MISC_FEATURE (1)..(1): Xaa at position 1 is gamma-Glu
  MOD_RES (2)..(7): There is a thioacetal bridge between the cysteines at positions 2 and 7
  MISC_FEATURE (11)..(11): Xaa at position 11 is Orn
  MISC_FEATURE (15)..(15): Xaa at position 15 is alpha-methyl-Phe
  MISC_FEATURE (22)..(22): Xaa at position 22 is N-methyl-Asp
  MOD_RES (26)..(26): The lysine at position 26 is attached to a fatty acid linker moiety according to the formula (gamma-Glu)2-CO-(CH2)18-CO2H
  MOD_RES (37)..(37): Tyr at position 37 is amidated

SEQ ID NO: 5 - protein, 37 aa, Artificial Sequence
  Synthetic Construct
  MISC_FEATURE (11)..(11): Xaa at position 11 is Orn
  MISC_FEATURE (15)..(15): Xaa at position 15 is alpha-methyl-Phe
  MISC_FEATURE (22)..(22): Xaa at position 22 is N-methyl-Asp
  MOD_RES (37)..(37): Tyr at position 37 is amidated
KCETATCATGXLAEXLVRSSNXFGPILPPTEVGSNTY

SEQ ID NO: 6 - protein, 37 aa, Artificial Sequence; identical to SEQ ID NO: 5
  Synthetic Construct
  MOD_RES (1)..(1): The lysine at position 1 is attached to a fatty acid linker moiety according to the formula (gamma-Glu)2-CO-(CH2)18-CO2H
  MOD_RES (2)..(7): There is a thioacetal bridge between the cysteines at positions 2 and 7
  MISC_FEATURE (11)..(11): Xaa at position 11 is Orn
  MISC_FEATURE (15)..(15): Xaa at position 15 is alpha-methyl-Phe
  MISC_FEATURE (22)..(22): Xaa at position 22 is N-methyl-Asp
  MOD_RES (37)..(37): Tyr at position 37 is amidated

SEQ ID NO: 7 - protein, 37 aa, Artificial Sequence
  Synthetic Construct
  MISC_FEATURE (11)..(11): Xaa at position 11 is Orn
  MISC_FEATURE (12)..(12): Xaa at position 12 is alpha-Methyl-Leu
  MOD_RES (37)..(37): Tyr at position 37 is amidated
KCETATCATGXXAEFLVRSSHNFGPILPPTEVGSNTY

SEQ ID NO: 8 - protein, 37 aa, Artificial Sequence; identical to SEQ ID NO: 7
  Synthetic Construct
  MOD_RES (1)..(1): The lysine at position 1 is attached to a fatty acid linker moiety according to the formula (gamma-Glu)2-CO-(CH2)18-CO2H
  MOD_RES (2)..(7): There is a thioacetal bridge between the cysteines at positions 2 and 7
  MISC_FEATURE (11)..(11): Xaa at position 11 is Orn
  MISC_FEATURE (12)..(12): Xaa at position 12 is alpha-Methyl-Leu
  MOD_RES (37)..(37): Tyr at position 37 is amidated

SEQ ID NO: 9 - protein, 37 aa, Artificial Sequence
  Synthetic Construct
  MISC_FEATURE (1)..(1): Xaa at position 1 is gamma-Glu
  MOD_RES (2)..(7): There is a thioacetal bridge between the cysteines at positions 2 and 7
  MOD_RES (26)..(26): The lysine at position 26 is attached to a fatty acid linker moiety according to the formula (AEEA)2-(gamma-Glu)-CO-(CH2)18-CO2H
  MOD_RES (37)..(37): Tyr at position 37 is amidated
XCNTATCATGKLAEFLVRSSNNFGPKLPPTEVGSNTY

SEQ ID NO: 10 - protein, 37 aa, Artificial Sequence; identical to SEQ ID NO: 9
  Synthetic Construct
  MISC_FEATURE (1)..(1): Xaa at position 1 is gamma-Glu
  MOD_RES (2)..(7): There is a thioacetal bridge between the cysteines at positions 2 and 7
  MOD_RES (26)..(26): The lysine at position 26 is attached to a fatty acid linker moiety according to the formula (gamma-Glu)-(AEEA)2-CO-(CH2)18-CO2H
  MOD_RES (37)..(37): Tyr at position 37 is amidated

SEQ ID NO: 11 - protein, 37 aa, Artificial Sequence; identical to SEQ ID NO: 9
  Synthetic Construct
  MISC_FEATURE (1)..(1): Xaa at position 1 is gamma-Glu
  MOD_RES (2)..(7): There is a thioacetal bridge between the cysteines at positions 2 and 7
  MOD_RES (26)..(26): The lysine at position 26 is attached to a fatty acid linker moiety according to the formula (gamma-Glu)2-AEEA-CO-(CH2)18-CO2H
  MOD_RES (37)..(37): Tyr at position 37 is amidated

SEQ ID NO: 12 - protein, 37 aa, Artificial Sequence
  Synthetic Construct
  MISC_FEATURE (1)..(1): Xaa at position 1 is gamma-Glu
  MOD_RES (2)..(7): There is a thioacetal bridge between the cysteines at positions 2 and 7
  MISC_FEATURE (11)..(11): Xaa at position 11 is Orn
  MOD_RES (26)..(26): The lysine at position 26 is attached to a fatty acid linker moiety according to the formula (AEEA)2-(gamma-Glu)-CO-(CH2)18-CO2H
  MOD_RES (37)..(37): Tyr at position 37 is amidated
XCNTATCATQXLAEFLVRSSNNFGPKLPPTEVGSNTY

SEQ ID NO: 13 - protein, 37 aa, Artificial Sequence
  Synthetic Construct
  MISC_FEATURE (1)..(1): Xaa at position 1 is gamma-Glu
  MOD_RES (2)..(7): There is a thioacetal bridge between the cysteines at positions 2 and 7
  MISC_FEATURE (11)..(11): Xaa at position 11 is Orn
  MOD_RES (26)..(26): The lysine at position 26 is attached to a fatty acid linker moiety according to the formula (gamma-Glu)2-CO-(CH2)18-CO2H
  MOD_RES (37)..(37): Tyr at position 37 is amidated
XCGTATCATGXLAEFLVRSSNNFGPKLPPTEVGSNTY

SEQ ID NO: 14 - protein, 37 aa, Artificial Sequence
  Synthetic Construct
  MISC_FEATURE (1)..(1): Xaa at position 1 is Lys or gamma-Glu
  MISC_FEATURE (3)..(3): Xaa at position 3 is Glu, Asn, or Gly
  MISC_FEATURE (10)..(10): Xaa at position 10 is Gly or Gln
  MISC_FEATURE (11)..(11): Xaa at position 11 is Orn or Lys
  MISC_FEATURE (12)..(12): Xaa at position 12 is Leu or alpha-methyl-Leu
  MISC_FEATURE (15)..(15): Xaa at position 15 is alpha-methyl-Phe or Phe
  MISC_FEATURE (21)..(21): Xaa at position 21 is Asn or His
  MISC_FEATURE (22)..(22): Xaa at position 22 is N-methyl-Asp, N-methyl-Asn, or Asn
  MISC_FEATURE (26)..(26): Xaa at position 26 is Ile or Lys
  MOD_RES (37)..(37): C-terminus is amidated
XCXTATCATXXXAEXLVRSSXXFGPXLPPTEVGSNTY

SEQ ID NO: 15 - protein, 37 aa, Artificial Sequence
  Synthetic Construct
  DISULFID (2)..(7)
  MOD_RES (37)..(37): Tyr at position 37 is amidated
KCNTATCATQRLANFLVHSSNNFGPILPPTNVGSNTY

SEQ ID NO: 16 - protein, 32 aa, Homo sapiens
  DISULFID (1)..(7)
  MOD_RES (32)..(32): Pro at position 32 is amidated
CGNLSTCMLGTYTQDFNKFHTFPQTAIGVGAP

SEQ ID NO: 17 - protein, 37 aa, Homo sapiens [sequence omitted]

SEQ ID NO: 18 - protein, 31 aa, Artificial Sequence
  Synthetic Construct
  MISC_FEATURE (2)..(2): Xaa at position 2 is Aib
  MOD_RES (20)..(20): The lysine at position 20 is attached to a fatty acid linker moiety according to the formula (2-[2-(2-Amino-ethoxy)-ethoxy]-acetyl)2-(gamma-Glu)-CO-(CH2)16-CO 2H
HXEGTFTSDVSSYLEGQAAKEFIAWLVRGRG

SEQ ID NO: 19 - protein, 34 aa, Artificial Sequence
  Synthetic Construct
  MISC_FEATURE (2)..(2): Xaa at position 2 is Aib
  MOD_RES (20)..(20): Lys at position 20 is chemically modified by conjugation of the epsilon-amino group of the Lys side chain with (2-[2-(2-amino-ethoxy)-ethoxy]-acetyl)2-(gamma-Glu)-CO-(CH2)18-CO 2H
  MOD_RES (34)..(34): Gly at position 34 is amidated
HXQGTFTSDYSKYLDEKKAKEFVEWLLEGGPSSG

SEQ ID NO: 20 - protein, 39 aa, Artificial Sequence
  Synthetic Construct
  MISC_FEATURE (2)..(2): Xaa at position 2 is Aib
  MISC_FEATURE (13)..(13): Xaa at position 13 is alpha-Methyl-Leu
  MOD_RES (17)..(17): Lys at position 17 is chemically modified by conjugation of the epsilon-amino group of the Lys side chain with (2-[2-(2-amino-ethoxy)-ethoxy]-acetyl)-(gamma-Glu)-CO-(CH2)18-CO2 H
  MISC_FEATURE (20)..(20): Xaa at position 20 is Aib
  MOD_RES (39)..(39): Ser at position 39 is amidated
YXQGTFTSDYSIXLDKKAQXAFIEYLLEGGPSSGAPPPS

SEQ ID NO: 21 - protein, 39 aa, Artificial Sequence
  Synthetic Construct
  MISC_FEATURE (2)..(2): Xaa at position 2 is Aib
  MISC_FEATURE (13)..(13): Xaa at position 13 is Aib
  MOD_RES (20)..(20): K at position 20 is chemically modified through conjugation to the epsilon-amino group of the K side-chain with (2-[2-(2-Amino-ethoxy)-ethoxy]-acetyl)2-(gamma-Glu)1-CO-(CH2)18-C O2H
  MOD_RES (39)..(39): Serine is amidated as a C-terminal primary amide
YXEGTFTSDYSIXLDKIAQKAFVQWLIAGGPSSGAPPPS

SEQ ID NO: 22 - protein, 37 aa, Artificial Sequence; identical to SEQ ID NO: 1
  Synthetic Construct
  MISC_FEATURE (1)..(1): Xaa at position 1 is gamma-Glu
  MISC_FEATURE (11)..(11): Xaa at position 11 is Orn
  MISC_FEATURE (15)..(15): Xaa at position 15 is alpha-Me-Phe
  MISC_FEATURE (22)..(22): Xaa at position 22 is N-Me-Asn
  MOD_RES (37)..(37): Tys at position 37 is amidated

SEQ ID NO: 23 - protein, 37 aa, Artificial Sequence; identical to SEQ ID NO: 1
  Synthetic Construct
  MISC_FEATURE (1)..(1): Xaa at position 1 is gamma-Glu
  MISC_FEATURE (11)..(11): Xaa at position 11 is Orn
  MISC_FEATURE (15)..(15): Xaa at position 15 is alpha-Me-Phe
  MISC_FEATURE (22)..(22): Xaa at position 22 is N-Me-Asp
  MOD_RES (37)..(37): Tys at position 37 is amidated

SEQ ID NO: 24 - protein, 37 aa, Artificial Sequence; identical to SEQ ID NO: 5
  Synthetic Construct
  MISC_FEATURE (11)..(11): Xaa at position 11 is Orn
  MISC_FEATURE (15)..(15): Xaa at position 15 is alpha-Me-Phe
  MISC_FEATURE (22)..(22): Xaa at position 22 is N-Me-Asp
  MOD_RES (37)..(37): Tys at position 37 is amidated

SEQ ID NO: 25 - protein, 37 aa, Artificial Sequence; identical to SEQ ID NO: 7
  Synthetic Construct
  MISC_FEATURE (11)..(11): Xaa at position 11 is Orn
  MISC_FEATURE (12)..(12): Xaa at position 12 is alpha-Me-Leu
  MOD_RES (37)..(37): Tys at position 37 is amidated